European Patent Specification EP 3 851 100 B1, published May 28, 2025. Title: METHODS OF TREATING CARDIOMYOPATHY, SYSTOLIC CARDIAC DYSFUNCTION AND THE SYMPTOMS OF CONGESTIVE HEART FAILURE WITH PROBENECID. Applicant: University of Cincinnati. Application EP12781543.9. The sequence listing filed with the application follows.

SEQUENCE LISTING (2 sequences)

SEQ ID NO: 1 - DNA, 18 bp, Mus musculus
ctactgctcaacatgctc

SEQ ID NO: 2 - DNA, 19 bp, Mus musculus
ctcatcaggtataccatcc